European Patent Specification EP 3 658 915 B1, published March 5, 2025. Title: New subpopulations of cancer associated fibroblasts as prognosis markers for immunotherapy treatments. Applicant: Institut Curie ISERM. The sequence listing filed with the application follows.

SEQUENCE LISTING (12 sequences)

SEQ ID NO: 1 - DNA, 20 bp, Artificial Sequence
  DPP4 Forward Primer
agtggcgtgttcaagtgtgg

SEQ ID NO: 2 - DNA, 22 bp, Artificial Sequence
  DPP4 reverse primer
caaggttgtcttctggagttgg

SEQ ID NO: 3 - DNA, 22 bp, Artificial Sequence
  OX40L forward primer
cctcgaattcaaagtatcaaag

SEQ ID NO: 4 - DNA, 21 bp, Artificial Sequence
  OX40L reverqse primer
gtgaggatgaaacctttctcc

SEQ ID NO: 5 - DNA, 20 bp, Artificial Sequence
  CD73 forward primer
ctcctctcaatcatgccgct

SEQ ID NO: 6 - DNA, 21 bp, Artificial Sequence
  CD73 reverse primer
tggattccattgttgcgttca

SEQ ID NO: 7 - DNA, 21 bp, Artificial Sequence
  PDL2 forward primer
acagtgctatctgaacctgtg

SEQ ID NO: 8 - DNA, 21 bp, Artificial Sequence
  PDL2 reverse primer
gtcatatcaggtcaccctggc

SEQ ID NO: 9 - DNA, 22 bp, Artificial Sequence
  B7H3 forward primer
ctggctttcgtgtgctggagaa

SEQ ID NO: 10 - DNA, 22 bp, Artificial Sequence
  B7H3 reverse primer
gctgtcagagtgtttcagaggc

SEQ ID NO: 11 - DNA, 20 bp, artificial
  JAM2 forward primer
cgccctgggctatcataagg

SEQ ID NO: 12 - DNA, 20 bp, artificial
  JAM2 reverse primer
caaaggagacactccgaccc